European Patent Application EP 4 403 184 A1, published July 24, 2024. Title: Pharmaceutical composition for use in treating decline in cognitive function. Applicant: 国立大学法人　琉球大学. The sequence listing filed with the application follows.

SEQUENCE LISTING (52 sequences)

SEQ ID NO: 1 - DNA, 2652 bp, Homo sapiens
  source 1..2652: mol_type = other DNA
  CDS 1..2652: protein_id = 50; translation = MQKIMHISVLLSPVLWGLIFGVSSNSIQIGGLFPRGADQEYSAFRVGMVQFSTSEFRLTPHIDNLEVANSFAVTNAFCSQFSRGVYAIFGFYDKKSVNTITSFCGTLHVSFITPSFPTDGTHPFVIQMRPDLKGALLSLIEYYQWDKFAYLYDSDRGLSTLQAVLDSAAEKKWQVTAINVGNINNDKKDEMYRSLFQDLELKKERRVILDCERDKVNDIVDQVITIGKHVKGYHYIIANLGFTDGDLLKIQFGGANVSGFQIVDYDDSLVSKFIERWSTLEEKEYPGAHTTTIKYTSALTYDAVQVMTEAFRNLRKQRIEISRRGNAGDCLANPAVPWGQGVEIERALKQVQVEGLSGNIKFDQNGKRINYTINIMELKTNGPRKIGYWSEVDKMVVTLTELPSGNDTSGLENKTVVVTTILESPYVMMKKNHEMLEGNERYEGYCVDLAAEIAKHCGFKYKLTIVGDGKYGARDADTKIWNGMVGELVYGKADIAIAPLTITLVREEVIDFSKPFMSLGISIMIKKPQKSKPGVFSFLDPLAYEIWMCIVFAYIGVSVVLFLVSRFSPYEWHTEEFEDGRETQSSESTNEFGIFNSLWFSLGAFMQQGCDISPRSLSGRIVGGVWWFFTLIIISSYTANLAAFLTVERMVSPIESAEDLSKQTEIAYGTLDSGSTKEFFRRSKIAVFDKMWTYMRSAEPSVFVRTTAEGVARVRKSKGKYAYLLESTMNEYIEQRKPCDTMKVGGNLDSKGYGIATPKGSSLRTPVNLAVLKLSEQGVLDKLKNKWWYDKGECGAKDSGSKEKTSALSLSNVAGVFYILVGGLGLAMLVALIEFCYKSRAEAKRMKVAKNAQNINPSSSQNSQNFATYKEGYNVYGIESVKI
atgcaaaagattatgcatatttctgtcctcctttctcctgttttatggggactgatttttggtgtctcttctaacagcatacagataggggggctatttcctaggggcgccgatcaagaatacagtgcatttcgagtagggatggttcagttttccacttcggagttcagactgacaccccacatcgacaatttggaggtggcaaacagcttcgcagtcactaatgctttctgctcccagttttcgagaggagtctatgctatttttggattttatgacaagaagtctgtaaataccatcacatcattttgcggaacactccacgtctccttcatcactcccagcttcccaacagatggcacacatccatttgtcattcagatgagacccgacctcaaaggagctctccttagcttgattgaatactatcaatgggacaagtttgcatacctctatgacagtgacagaggcttatcaacactgcaagctgtgctggattctgctgctgaaaagaaatggcaagtgactgctatcaatgtgggaaacattaacaatgacaagaaagatgagatgtaccgatcactttttcaagatctggagttaaaaaaggaacggcgtgtaattctggactgtgaaagggataaagtaaacgacattgtagaccaggttattaccattggaaaacatgttaaagggtaccactacatcattgcaaatctgggatttactgatggagacctattaaaaatccagtttggaggtgcaaatgtctctggatttcagatagtggactatgatgattcgttggtatctaaatttatagaaagatggtcaacactggaagaaaaagaataccctggagctcacacaacaacaattaagtatacttctgctctgacctatgatgccgttcaagtgatgactgaagccttccgcaacctaaggaagcaaagaattgaaatctcccgaagggggaatgcaggagactgtctggcaaacccagcagtgccctggggacaaggtgtagaaatagaaagggccctcaaacaggttcaggttgaaggtctctcaggaaatataaagtttgaccagaatggaaaaagaataaactatacaattaacatcatggagctcaaaactaatgggccccggaagattggctactggagtgaagtggacaaaatggttgttacccttactgagctcccttctggaaatgacacctctgggcttgagaataagactgttgttgtcaccacaattttggaatctccgtatgttatgatgaagaaaaatcatgaaatgcttgaaggcaatgagcgctatgagggctactgtgttgacctggctgcagaaatcgccaaacattgtgggttcaagtacaagttgacaattgttggtgatggcaagtatggggccagggatgcagacacgaaaatttggaatgggatggttggagaacttgtatatgggaaagctgatattgcaattgctccattaactattacccttgtgagagaagaggtgattgacttctcaaagcccttcatgagcctcgggatatctatcatgatcaagaagcctcagaagtccaaaccaggagtgttttcctttcttgatcctttagcctatgagatctggatgtgcattgtttttgcctacattggggtcagtgtagttttattcctggtcagcagatttagcccctacgagtggcacactgaggagtttgaagatggaagagaaacacaaagtagtgaatcaactaatgaatttgggatttttaatagtctctggttttccttgggtgcctttatgcagcaaggatgcgatatttcgccaagatccctctctgggcgcattgttggaggtgtgtggtggttctttaccctgatcataatctcctcctacacggctaacttagctgccttcctgactgtagagaggatggtgtctcccatcgaaagtgctgaggatctttctaagcaaacagaaattgcttatggaacattagactctggctccactaaagagtttttcaggagatctaaaattgcagtgtttgataaaatgtggacctacatgcggagtgcggagccctctgtgtttgtgaggactacggccgaaggggtggctagagtgcggaagtccaaagggaaatatgcctacttgttggagtccacgatgaacgagtacattgagcaaaggaagccttgcgacaccatgaaagttggtggaaacctggattccaaaggctatggcatcgcaacacctaaaggatcctcattaagaaccccagtaaatcttgcagtattgaaactcagtgagcaaggcgtcttagacaagctgaaaaacaaatggtggtacgataaaggtgaatgtggagccaaggactctggaagtaaggaaaagaccagtgccctcagtctgagcaacgttgctggagtattctacatccttgtcgggggccttggtttggcaatgctggtggctttgattgagttctgttacaagtcaagggccgaggcgaaacgaatgaaggtggcaaagaatgcacagaatattaacccatcttcctcgcagaattcacagaattttgcaacttataaggaaggttacaacgtatatggcatcgaaagtgttaaaatttag

SEQ ID NO: 2 - protein, 883 aa, Homo sapiens
MQKIMHISVLLSPVLWGLIFGVSSNSIQIGGLFPRGADQEYSAFRVGMVQFSTSEFRLTPHIDNLEVANSFAVTNAFCSQFSRGVYAIFGFYDKKSVNTITSFCGTLHVSFITPSFPTDGTHPFVIQMRPDLKGALLSLIEYYQWDKFAYLYDSDRGLSTLQAVLDSAAEKKWQVTAINVGNINNDKKDEMYRSLFQDLELKKERRVILDCERDKVNDIVDQVITIGKHVKGYHYIIANLGFTDGDLLKIQFGGANVSGFQIVDYDDSLVSKFIERWSTLEEKEYPGAHTTTIKYTSALTYDAVQVMTEAFRNLRKQRIEISRRGNAGDCLANPAVPWGQGVEIERALKQVQVEGLSGNIKFDQNGKRINYTINIMELKTNGPRKIGYWSEVDKMVVTLTELPSGNDTSGLENKTVVVTTILESPYVMMKKNHEMLEGNERYEGYCVDLAAEIAKHCGFKYKLTIVGDGKYGARDADTKIWNGMVGELVYGKADIAIAPLTITLVREEVIDFSKPFMSLGISIMIKKPQKSKPGVFSFLDPLAYEIWMCIVFAYIGVSVVLFLVSRFSPYEWHTEEFEDGRETQSSESTNEFGIFNSLWFSLGAFMQQGCDISPRSLSGRIVGGVWWFFTLIIISSYTANLAAFLTVERMVSPIESAEDLSKQTEIAYGTLDSGSTKEFFRRSKIAVFDKMWTYMRSAEPSVFVRTTAEGVARVRKSKGKYAYLLESTMNEYIEQRKPCDTMKVGGNLDSKGYGIATPKGSSLRTPVNLAVLKLSEQGVLDKLKNKWWYDKGECGAKDSGSKEKTSALSLSNVAGVFYILVGGLGLAMLVALIEFCYKSRAEAKRMKVAKNAQNINPSSSQNSQNFATYKEGYNVYGIESVKI

SEQ ID NO: 3 - protein, 883 aa, Homo sapiens
MQKIMHISVLLSPVLWGLIFGVSSNSIQIGGLFPRGADQEYSAFRVGMVQFSTSEFRLTPHIDNLEVANSFAVTNAFCSQFSRGVYAIFGFYDKKSVNTITSFCGTLHVSFITPSFPTDGTHPFVIQMRPDLKGALLSLIEYYQWDKFAYLYDSDRGLSTLQAVLDSAAEKKWQVTAINVGNINNDKKDEMYRSLFQDLELKKERRVILDCERDKVNDIVDQVITIGKHVKGYHYIIANLGFTDGDLLKIQFGGANVSGFQIVDYDDSLVSKFIERWSTLEEKEYPGAHTTTIKYTSALTYDAVQVMTEAFRNLRKQRIEISRRGNAGDCLANPAVPWGQGVEIERALKQVQVEGLSGNIKFDQNGKRINYTINIMELKTNGPRKIGYWSEVDKMVVTLTELPSGNDTSGLENKTVVVTTILESPYVMMKKNHEMLEGNERYEGYCVDLAAEIAKHCGFKYKLTIVGDGKYGARDADTKIWNGMVGELVYGKADIAIAPLTITLVREEVIDFSKPFMSLGISIMIKKPQKSKPGVFSFLDPLAYEIWMCIVFAYIGVSVVLFLVSRFSPYEWHTEEFEDGRETQSSESTNEFGIFNSLWFSLGAFMRQGCDISPRSLSGRIVGGVWWFFTLIIISSYTANLAAFLTVERMVSPIESAEDLSKQTEIAYGTLDSGSTKEFFRRSKIAVFDKMWTYMRSAEPSVFVRTTAEGVARVRKSKGKYAYLLESTMNEYIEQRKPCDTMKVGGNLDSKGYGIATPKGSSLRTPVNLAVLKLSEQGVLDKLKNKWWYDKGECGAKDSGSKEKTSALSLSNVAGVFYILVGGLGLAMLVALIEFCYKSRAEAKRMKVAKNAQNINPSSSQNSQNFATYKEGYNVYGIESVKI

SEQ ID NO: 4 - DNA, 2721 bp, Homo sapiens
  source 1..2721: mol_type = other DNA
  CDS 1..2721: protein_id = 51; translation = MQHIFAFFCTGFLGAVVGANFPNNIQIGGLFPNQQSQEHAAFRFALSQLTEPPKLLPQIDIVNISDSFEMTYRFCSQFSKGVYAIFGFYERRTVNMLTSFCGALHVCFITPSFPVDTSNQFVLQLRPELQDALISIIDHYKWQKFVYIYDADRGLSVLQKVLDTAAEKNWQVTAVNILTTTEEGYRMLFQDLEKKKERLVVVDCESERLNAILGQIIKLEKNGIGYHYILANLGFMDIDLNKFKESGANVTGFQLVNYTDTIPAKIMQQWKNSDARDHTRVDWKRPKYTSALTYDGVKVMAEAFQSLRRQRIDISRRGNAGDCLANPAVPWGQGIDIQRALQQVRFEGLTGNVQFNEKGRRTNYTLHVIEMKHDGIRKIGYWNEDDKFVPAATDAQAGGDNSSVQNRTYIVTTILEDPYVMLKKNANQFEGNDRYEGYCVELAAEIAKHVGYSYRLEIVSDGKYGARDPDTKAWNGMVGELVYGRADVAVAPLTITLVREEVIDFSKPFMSLGISIMIKKPQKSKPGVFSFLDPLAYEIWMCIVFAYIGVSVVLFLVSRFSPYEWHSEEFEEGRDQTTSDQSNEFGIFNSLWFSLGAFMQQGCDISPRSLSGRIVGGVWWFFTLIIISSYTANLAAFLTVERMVSPIESAEDLAKQTEIAYGTLEAGSTKEFFRRSKIAVFEKMWTYMKSAEPSVFVRTTEEGMIRVRKSKGKYAYLLESTMNEYIEQRKPCDTMKVGGNLDSKGYGIATPKGSALRNPVNLAVLKLNEQGLLDKLKNKWWYDKGECGSGGGDSKDKTSALSLSNVAGVFYILIGGLGLAMLVALIEFCYKSRSESKRMKGFCLIPQQSINEAIRTSTLPRNSGAGASSGGSGENGRVVSHDFPKSMQSIPCMSHSSGMPLGATGL
atgcagcacatttttgccttcttctgcaccggtttcctaggcgcggtagtaggtgccaatttccccaacaatatccagatcgggggattatttccaaaccagcagtcacaggaacatgctgcttttagatttgctttgtcgcaactcacagagcccccgaagctgctcccccagattgatattgtgaacatcagcgacagctttgagatgacctatagattctgttcccagttctccaaaggagtctatgccatctttgggttttatgaacgtaggactgtcaacatgctgacctccttttgtggggccctccacgtctgcttcattacgccgagctttcccgttgatacatccaatcagtttgtccttcagctgcgccctgaactgcaggatgccctcatcagcatcattgaccattacaagtggcagaaatttgtctacatttatgatgccgaccggggcttatccgtcctgcagaaagtcctggatacagctgctgagaagaactggcaggtgacagcagtcaacattttgacaaccacagaggagggataccggatgctctttcaggacctggagaagaaaaaggagcggctggtggtggtggactgtgaatcagaacgcctcaatgctatcttgggccagattataaagctagagaagaatggcatcggctaccactacattcttgcaaatctgggcttcatggacattgacttaaacaaattcaaggagagtggcgccaatgtgacaggtttccagctggtgaactacacagacactattccggccaagatcatgcagcagtggaagaatagtgatgctcgagaccacacacgggtggactggaagagacccaagtacacctctgcgctcacctacgatggggtgaaggtgatggctgaggctttccagagcctgcggaggcagagaattgatatatctcgccgggggaatgctggggattgtctggctaacccagctgttccctggggccaagggatcgacatccagagagctctgcagcaggtgcgatttgaaggtttaacaggaaacgtgcagtttaatgagaaaggacgccggaccaactacacgctccacgtgattgaaatgaaacatgacggcatccgaaagattggttactggaatgaagatgataagtttgtccctgcagccaccgatgcccaagctgggggcgataattcaagtgttcagaacagaacatacatcgtcacaacaatcctagaagatccttatgtgatgctcaagaagaacgccaatcagtttgagggcaatgaccgttacgagggctactgtgtagagctggcggcagagattgccaagcacgtgggctactcctaccgtctggagattgtcagtgatggaaaatacggagcccgagaccctgacacgaaggcctggaatggcatggtgggagagctggtctatggaagagcagatgtggctgtggctcccttaactatcactttggtccgggaagaagttatagatttctccaaaccatttatgagtttggggatctccatcatgattaaaaaaccacagaaatccaagccgggtgtcttctccttccttgatcctttggcttatgagatttggatgtgcattgtttttgcctacattggagtgagtgttgtcctcttcctggtcagccgcttcagtccctatgaatggcacagtgaagagtttgaggaaggacgggaccagacaaccagtgaccagtccaatgagtttgggatattcaacagtttgtggttctccctgggagccttcatgcagcaaggatgtgacatttctcccaggtccctgtctggtcgcatcgttggtggcgtctggtggttcttcaccttaatcatcatctcctcatatacagccaatctggccgccttcctgaccgtggagaggatggtgtctcccattgagagtgcagaggacctagcgaagcagacagaaattgcctacgggacgctggaagcaggatctactaaggagttcttcaggaggtctaaaattgctgtgtttgagaagatgtggacatacatgaagtcagcagagccatcagtttttgtgcggaccacagaggaggggatgattcgagtgaggaaatccaaaggcaaatatgcctacctcctggagtccaccatgaatgagtacattgagcagcggaaaccctgtgacaccatgaaggtgggaggtaacttggattccaaaggctatggcattgcaacacccaaggggtctgccctgagaaatccagtaaacctggcagtgttaaaactgaacgagcaggggcttttggacaaattgaaaaacaaatggtggtacgacaagggcgagtgcggcagcgggggaggtgattccaaggacaagacaagcgctctgagcctcagcaatgtggcaggcgtgttctacatcctgatcggaggacttggactagccatgctggttgccttaatcgagttctgctacaaatcccgtagtgaatccaagcggatgaagggtttttgtttgatcccacagcaatccatcaacgaagccatacggacatcgaccctcccccgcaacagcggggcaggagccagcagcggcggcagtggagagaatggtcgggtggtcagccatgacttccccaagtccatgcaatcgattccttgcatgagccacagttcagggatgcccttgggagccacgggattgtaa

SEQ ID NO: 5 - protein, 906 aa, Homo sapiens
MQHIFAFFCTGFLGAVVGANFPNNIQIGGLFPNQQSQEHAAFRFALSQLTEPPKLLPQIDIVNISDSFEMTYRFCSQFSKGVYAIFGFYERRTVNMLTSFCGALHVCFITPSFPVDTSNQFVLQLRPELQDALISIIDHYKWQKFVYIYDADRGLSVLQKVLDTAAEKNWQVTAVNILTTTEEGYRMLFQDLEKKKERLVVVDCESERLNAILGQIIKLEKNGIGYHYILANLGFMDIDLNKFKESGANVTGFQLVNYTDTIPAKIMQQWKNSDARDHTRVDWKRPKYTSALTYDGVKVMAEAFQSLRRQRIDISRRGNAGDCLANPAVPWGQGIDIQRALQQVRFEGLTGNVQFNEKGRRTNYTLHVIEMKHDGIRKIGYWNEDDKFVPAATDAQAGGDNSSVQNRTYIVTTILEDPYVMLKKNANQFEGNDRYEGYCVELAAEIAKHVGYSYRLEIVSDGKYGARDPDTKAWNGMVGELVYGRADVAVAPLTITLVREEVIDFSKPFMSLGISIMIKKPQKSKPGVFSFLDPLAYEIWMCIVFAYIGVSVVLFLVSRFSPYEWHSEEFEEGRDQTTSDQSNEFGIFNSLWFSLGAFMQQGCDISPRSLSGRIVGGVWWFFTLIIISSYTANLAAFLTVERMVSPIESAEDLAKQTEIAYGTLEAGSTKEFFRRSKIAVFEKMWTYMKSAEPSVFVRTTEEGMIRVRKSKGKYAYLLESTMNEYIEQRKPCDTMKVGGNLDSKGYGIATPKGSALRNPVNLAVLKLNEQGLLDKLKNKWWYDKGECGSGGGDSKDKTSALSLSNVAGVFYILIGGLGLAMLVALIEFCYKSRSESKRMKGFCLIPQQSINEAIRTSTLPRNSGAGASSGGSGENGRVVSHDFPKSMQSIPCMSHSSGMPLGATGL

SEQ ID NO: 6 - DNA, 2685 bp, Homo sapiens
  source 1..2685: mol_type = other DNA
  CDS 1..2685: protein_id = 52; translation = MARQKKMGQSVLRAVFFLVLGLLGHSHGGFPNTISIGGLFMRNTVQEHSAFRFAVQLYNTNQNTTEKPFHLNYHVDHLDSSNSFSVTNAFCSQFSRGVYAIFGFYDQMSMNTLTSFCGALHTSFVTPSFPTDADVQFVIQMRPALKGAILSLLGHYKWEKFVYLYDTERGFSILQAIMEAAVQNNWQVTARSVGNIKDVQEFRRIIEEMDRRQEKRYLIDCEVERINTILEQVVILGKHSRGYHYMLANLGFTDILLERVMHGGANITGFQIVNNENPMVQQFIQRWVRLDEREFPEAKNAPLKYTSALTHDAILVIAEAFRYLRRQRVDVSRRGSAGDCLANPAVPWSQGIDIERALKMVQVQGMTGNIQFDTYGRRTNYTIDVYEMKVSGSRKAGYWNEYERFVPFSDQQISNDSASSENRTIVVTTILESPYVMYKKNHEQLEGNERYEGYCVDLAYEIAKHVRIKYKLSIVGDGKYGARDPETKIWNGMVGELVYGRADIAVAPLTITLVREEVIDFSKPFMSLGISIMIKKPQKSKPGVFSFLDPLAYEIWMCIVFAYIGVSVVLFLVSRFSPYEWHLEDNNEEPRDPQSPPDPPNEFGIFNSLWFSLGAFMQQGCDISPRSLSGRIVGGVWWFFTLIIISSYTANLAAFLTVERMVSPIESAEDLAKQTEIAYGTLDSGSTKEFFRRSKIAVYEKMWSYMKSAEPSVFTKTTADGVARVRKSKGKFAFLLESTMNEYIEQRKPCDTMKVGGNLDSKGYGVATPKGSALRTPVNLAVLKLSEQGILDKLKNKWWYDKGECGAKDSGSKDKTSALSLSNVAGVFYILVGGLGLAMMVALIEFCYKSRAESKRMKLTKNTQNFKPAPATNTQNYATYREGYNVYGTESVKI
atggccaggcagaagaaaatggggcaaagcgtgctccgggcggtcttctttttagtcctggggcttttgggtcattctcacggaggattccccaacaccatcagcataggtggacttttcatgagaaacacagtgcaggagcacagcgctttccgctttgccgtgcagttatacaacaccaaccagaacaccaccgagaagcccttccatttgaattaccacgtagatcacttggattcctccaatagtttttccgtgacaaatgctttctgctcccagttctcgagaggggtgtatgccatctttggattctatgaccagatgtcaatgaacaccctgacctccttctgtggggccctgcacacatcctttgttacgcctagcttccccactgacgcagatgtgcagtttgtcatccagatgcgcccagccttgaagggcgctattctgagtcttctgggtcattacaagtgggagaagtttgtgtacctctatgacacagaacgaggattttccatcctccaagcgattatggaagcagcagtgcaaaacaactggcaagtaacagcaaggtctgtgggaaacataaaggacgtccaagaattcaggcgcatcattgaagaaatggacaggaggcaggaaaagcgatacttgattgactgcgaagtcgaaaggattaacacaattttggaacaggttgtgatcctagggaaacactcaagaggttatcactacatgctcgctaacctgggttttactgatattttactggaaagagtcatgcatgggggagccaacattacaggtttccagattgtcaacaatgaaaaccctatggttcagcagttcatacagcgctgggtgaggctggatgaaagggaattccctgaagccaagaatgcaccactaaagtatacatctgcattgacacacgacgcaatactggtcatagcagaagctttccgctacctgaggaggcagcgagtagatgtgtcccggagaggaagtgctggagactgcttagcaaatcctgctgtgccctggagtcaaggaattgatattgagagagctctgaaaatggtgcaagtacaaggaatgactggaaatattcaatttgacacttatggacgtaggacaaattataccatcgatgtgtatgaaatgaaagtcagtggctctcgaaaagctggctactggaatgagtatgaaaggtttgtgcctttctcagatcagcaaatcagcaatgacagtgcatcctcagagaatcggaccatagtagtgactaccattctggaatcaccatatgtaatgtacaagaagaaccatgagcaactggaaggaaatgaacgatatgaaggctattgtgtagacctagcctatgaaatagccaaacatgtaaggatcaaatacaaattgtccatcgttggtgacgggaaatatggtgcaagggatccagagactaaaatatggaacggcatggttggggaacttgtctatgggagagctgatatagctgttgctccactcactataacattggtccgtgaagaagtcatagatttttcaaagccattcatgagcctgggcatctccatcatgataaagaagcctcagaaatcaaaaccaggcgtattctcatttctggatcccctggcttatgaaatctggatgtgcattgtctttgcttacattggagtcagcgtagttcttttcctagtcagcaggttcagtccttatgaatggcacttggaagacaacaatgaagaacctcgtgacccacaaagtcctcctgatcctccaaatgaatttggaatatttaacagtctttggttttccttgggtgcctttatgcagcaaggatgtgatatttctccaagatcactctccgggcgcattgttggaggggtttggtggttcttcaccctgatcataatttcttcctatactgccaatctcgctgctttcctgactgtggagaggatggtttctcccatagagagtgctgaagacttagctaaacagactgaaattgcatatgggaccctggactccggttcaacaaaagaatttttcagaagatccaaaattgctgtgtacgagaaaatgtggtcttacatgaaatcagcggagccatctgtgtttaccaaaacaacagcagacggagtggcccgagtgcgaaagtccaagggaaagttcgccttcctgctggagtcaaccatgaatgagtacattgagcagagaaaaccatgtgatacgatgaaagttggtggaaatctggattccaaaggctatggtgtggcaacccctaaaggctcagcattaagaacgcctgtaaaccttgcagtattgaaactcagtgaacaaggcatcttagacaagctgaaaaacaaatggtggtacgataagggggaatgtggagccaaggactccgggagtaaggacaagaccagcgctctgagcctgagcaatgtggcaggcgttttctatatacttgtcggaggtctggggctggccatgatggtggctttgatagaattctgttacaaatcacgggcagagtccaaacgcatgaaactcacaaagaacacccaaaactttaagcctgctcctgccaccaacactcagaattatgctacatacagagaaggctacaacgtgtatggaacagagagtgttaagatctag

SEQ ID NO: 7 - protein, 894 aa, Homo sapiens
MARQKKMGQSVLRAVFFLVLGLLGHSHGGFPNTISIGGLFMRNTVQEHSAFRFAVQLYNTNQNTTEKPFHLNYHVDHLDSSNSFSVTNAFCSQFSRGVYAIFGFYDQMSMNTLTSFCGALHTSFVTPSFPTDADVQFVIQMRPALKGAILSLLGHYKWEKFVYLYDTERGFSILQAIMEAAVQNNWQVTARSVGNIKDVQEFRRIIEEMDRRQEKRYLIDCEVERINTILEQVVILGKHSRGYHYMLANLGFTDILLERVMHGGANITGFQIVNNENPMVQQFIQRWVRLDEREFPEAKNAPLKYTSALTHDAILVIAEAFRYLRRQRVDVSRRGSAGDCLANPAVPWSQGIDIERALKMVQVQGMTGNIQFDTYGRRTNYTIDVYEMKVSGSRKAGYWNEYERFVPFSDQQISNDSASSENRTIVVTTILESPYVMYKKNHEQLEGNERYEGYCVDLAYEIAKHVRIKYKLSIVGDGKYGARDPETKIWNGMVGELVYGRADIAVAPLTITLVREEVIDFSKPFMSLGISIMIKKPQKSKPGVFSFLDPLAYEIWMCIVFAYIGVSVVLFLVSRFSPYEWHLEDNNEEPRDPQSPPDPPNEFGIFNSLWFSLGAFMQQGCDISPRSLSGRIVGGVWWFFTLIIISSYTANLAAFLTVERMVSPIESAEDLAKQTEIAYGTLDSGSTKEFFRRSKIAVYEKMWSYMKSAEPSVFTKTTADGVARVRKSKGKFAFLLESTMNEYIEQRKPCDTMKVGGNLDSKGYGVATPKGSALRTPVNLAVLKLSEQGILDKLKNKWWYDKGECGAKDSGSKDKTSALSLSNVAGVFYILVGGLGLAMMVALIEFCYKSRAESKRMKLTKNTQNFKPAPATNTQNYATYREGYNVYGTESVKI

SEQ ID NO: 8 - DNA, 2709 bp, Homo sapiens
  source 1..2709: mol_type = other DNA
  CDS 1..2709
atgaggattatttccagacagattgtcttgttattttctggattttggggactcgccatgggagcctttccgagcagcgtgcaaataggtggtctcttcatccgaaacacagatcaggaatacactgcttttcgattagcaatttttcttcataacaccagccccaatgcgtcggaagctccttttaatttggtacctcatgtggacaacattgagacagccaacagttttgctgtaacaaacgccttctgttcccagtattctagaggagtatttgccatttttggactctatgataagaggtcggtacataccttgacctcattctgcagcgccttacatatctccctcatcacaccaagtttccctactgagggggagagccagtttgtgctgcaactaagaccttcgttacgaggagcactcttgagtttgctggatcactacgaatggaactgttttgtcttcctgtatgacacagacaggggatactcgatactccaagctattatggaaaaagcaggacaaaatggttggcatgtcagcgctatatgtgtggaaaattttaatgatgtcagctataggcaacttctagaagaacttgacagaagacaagagaagaagtttgtaatagactgtgagatagagagacttcaaaacatattagaacagattgtaagtgttggaaagcatgttaaaggctaccattatatcattgcaaacttgggattcaaggatatttctcttgagaggtttatacatggtggagccaatgttactggattccagttggtggattttaatacacctatggtaatcaaactaatggatcgctggaagaaactagatcagagagagtatccaggatctgagactcctccaaagtacacctctgctctgacttatgatggagtccttgtgatggctgaaactttccgaagtcttaggaggcagaaaattgatatctcaaggagaggaaatgctggggattgtctggcaaatcctgctgctccatggggccagggaattgacatggagaggacactcaaacaggttcgaattcaagggctgacagggaatgttcagtttgaccactatggacgtagagtcaattacacaatggatgtgtttgagctgaaaagcacaggacctagaaaggttggttactggaatgatatggataagttagtcttgattcaagatgtaccaactcttggcaatgacacagctgctattgagaacagaacagtggttgtaaccacaattatggaatccccatatgttatgtacaagaaaaatcatgaaatgtttgaaggaaatgacaagtatgaaggatactgtgtagatttggcatctgaaattgcaaaacatattggtatcaagtataaaattgccattgtccctgatggaaaatatggagcaagggatgcagacacaaaaatctggaatgggatggtaggagaacttgtttatgggaaagcagagattgctattgcccctctgacaatcactttggtacgagaggaggtcattgacttttctaagcccttcatgagtttgggcatatctatcatgatcaaaaagcctcagaaatccaaaccaggagtgttttccttcttggatcctctggcctatgagatttggatgtgcatagtctttgcctacattggtgtcagcgtggtcttattcctagttagtagatttagtccatatgagtggcacacagaagagccagaggacggaaaggaaggacccagcgaccagcctcccaatgagtttggcatctttaacagcctctggttttccctgggtgcttttatgcagcaaggatgtgacatttcacccagatccctctcaggtcgaattgttggaggtgtttggtggttctttacactcatcattatatcatcttatactgctaacctcgctgctttcctgacggttgagcgaatggtctctcccatagaaagtgcagaagacctggccaaacaaacagaaattgcctatggaacactggattcaggatcaacaaaagaattcttcagaagatcaaaaatagcagtgtatgaaaagatgtggacctacatgcgatcagcagagccatcagtattcactaggactacagctgagggagtagctcgtgtccgcaaatccaagggcaaatttgcctttctcctggagtccactatgaatgaatacattgagcagcgaaagccatgtgacacgatgaaagtgggaggaaatctggattccaaaggctatggagtagcaacgcccaagggttcctcattaagaactcctgtaaaccttgccgttttgaaactcagtgaggcaggcgtcttagacaagctgaaaaacaaatggtggtacgataaaggtgaatgtggacccaaggactctggaagcaaggacaagacgagtgccttgagcctgagcaatgtagcaggcgtcttctacattctggttggcggcttgggcttggcaatgctggtggctttgatagagttctgttacaagtccagggcagaagcgaagagaatgaagctgaccttttctgaagccataagaaacaaagccagattatccatcactgggagtgtgggagagaatggccgcgtcttgacgcctgactgcccaaaggctgtacacactggaactgcaatcagacaaagttcaggattggctgtcattgcatcggacctaccataa

SEQ ID NO: 9 - protein, 902 aa, Homo sapiens
MRIISRQIVLLFSGFWGLAMGAFPSSVQIGGLFIRNTDQEYTAFRLAIFLHNTSPNASEAPFNLVPHVDNIETANSFAVTNAFCSQYSRGVFAIFGLYDKRSVHTLTSFCSALHISLITPSFPTEGESQFVLQLRPSLRGALLSLLDHYEWNCFVFLYDTDRGYSILQAIMEKAGQNGWHVSAICVENFNDVSYRQLLEELDRRQEKKFVIDCEIERLQNILEQIVSVGKHVKGYHYIIANLGFKDISLERFIHGGANVTGFQLVDFNTPMVIKLMDRWKKLDQREYPGSETPPKYTSALTYDGVLVMAETFRSLRRQKIDISRRGNAGDCLANPAAPWGQGIDMERTLKQVRIQGLTGNVQFDHYGRRVNYTMDVFELKSTGPRKVGYWNDMDKLVLIQDVPTLGNDTAAIENRTVVVTTIMESPYVMYKKNHEMFEGNDKYEGYCVDLASEIAKHIGIKYKIAIVPDGKYGARDADTKIWNGMVGELVYGKAEIAIAPLTITLVREEVIDFSKPFMSLGISIMIKKPQKSKPGVFSFLDPLAYEIWMCIVFAYIGVSVVLFLVSRFSPYEWHTEEPEDGKEGPSDQPPNEFGIFNSLWFSLGAFMQQGCDISPRSLSGRIVGGVWWFFTLIIISSYTANLAAFLTVERMVSPIESAEDLAKQTEIAYGTLDSGSTKEFFRRSKIAVYEKMWTYMRSAEPSVFTRTTAEGVARVRKSKGKFAFLLESTMNEYIEQRKPCDTMKVGGNLDSKGYGVATPKGSSLRTPVNLAVLKLSEAGVLDKLKNKWWYDKGECGPKDSGSKDKTSALSLSNVAGVFYILVGGLGLAMLVALIEFCYKSRAEAKRMKLTFSEAIRNKARLSITGSVGENGRVLTPDCPKAVHTGTAIRQSSGLAVIASDLP

SEQ ID NO: 10 - DNA, 16 bp, synthetic construct
  misc_feature 1..16: note = beta-actin forward
  source 1..16: mol_type = other DNA
acagcttcacacagct

SEQ ID NO: 11 - DNA, 18 bp, synthetic construct
  misc_feature 1..18: note = beta-actin reverse
  source 1..18: mol_type = other DNA
tgcgagtggccatctcct

SEQ ID NO: 12 - DNA, 20 bp, synthetic construct
  misc_feature 1..20: note = GluA1 forward
  source 1..20: mol_type = other DNA
ctgtgaatcagaacgcctca

SEQ ID NO: 13 - DNA, 20 bp, synthetic construct
  misc_feature 1..20: note = GluA1 reverse
  source 1..20: mol_type = other DNA
ggaaacctgtcacattggct

SEQ ID NO: 14 - DNA, 18 bp, synthetic construct
  misc_feature 1..18: note = GluA2 forward
  source 1..18: mol_type = other DNA
ccctggagcacacagcga

SEQ ID NO: 15 - DNA, 20 bp, synthetic construct
  misc_feature 1..20: note = GluA2 reverse
  source 1..20: mol_type = other DNA
ctgcttccgaagattgcgga

SEQ ID NO: 16 - DNA, 21 bp, synthetic construct
  misc_feature 1..21: note = GluA3 forward
  source 1..21: mol_type = other DNA
gtgcagttatacaaccaacca

SEQ ID NO: 17 - DNA, 23 bp, synthetic construct
  misc_feature 1..23: note = GluA3 reverse
  source 1..23: mol_type = other DNA
gagcagaaagcattagtcacaga

SEQ ID NO: 18 - DNA, 15 bp, synthetic construct
  misc_feature 1..15: note = GluA4 forward
  source 1..15: mol_type = other DNA
ggctcagtgcactca

SEQ ID NO: 19 - DNA, 17 bp, synthetic construct
  misc_feature 1..17: note = GluA4 reverse
  source 1..17: mol_type = other DNA
ctctgcagtgcgacaca

SEQ ID NO: 20 - DNA, 14 bp, synthetic construct
  misc_feature 1..14: note = GluN1 forward
  source 1..14: mol_type = other DNA
ctcgcatgcaagac

SEQ ID NO: 21 - DNA, 20 bp, synthetic construct
  misc_feature 1..20: note = GluN1 reverse
  source 1..20: mol_type = other DNA
tgtcttatccaggtcttcca

SEQ ID NO: 22 - DNA, 20 bp, synthetic construct
  misc_feature 1..20: note = GluN2A forward
  source 1..20: mol_type = other DNA
gggtcacagagcaacatgct

SEQ ID NO: 23 - DNA, 21 bp, synthetic construct
  misc_feature 1..21: note = GluN2A reverse
  source 1..21: mol_type = other DNA
agctctttttgggtgagtcca

SEQ ID NO: 24 - DNA, 20 bp, synthetic construct
  misc_feature 1..20: note = GluN2B forward
  source 1..20: mol_type = other DNA
gtgagagctcctttgccaac

SEQ ID NO: 25 - DNA, 17 bp, synthetic construct
  misc_feature 1..17: note = GluN2B reverse
  source 1..17: mol_type = other DNA
tcagagagcgaactgct

SEQ ID NO: 26 - DNA, 20 bp, synthetic construct
  misc_feature 1..20: note = GluN2C forward
  source 1..20: mol_type = other DNA
aaggccttttgtcattgtgg

SEQ ID NO: 27 - DNA, 20 bp, synthetic construct
  misc_feature 1..20: note = GluN2C reverse
  source 1..20: mol_type = other DNA
cttgaggatgtcgatgcaga

SEQ ID NO: 28 - DNA, 20 bp, synthetic construct
  misc_feature 1..20: note = GluN2D forward
  source 1..20: mol_type = other DNA
gactactccttcaatgagga

SEQ ID NO: 29 - DNA, 20 bp, synthetic construct
  misc_feature 1..20: note = GluN2D reverse
  source 1..20: mol_type = other DNA
gttcccagctgcccaccact

SEQ ID NO: 30 - DNA, 19 bp, synthetic construct
  misc_feature 1..19: note = GluN3A forward
  source 1..19: mol_type = other DNA
ccagtcagggtttcacaga

SEQ ID NO: 31 - DNA, 20 bp, synthetic construct
  misc_feature 1..20: note = GluN3A reverse
  source 1..20: mol_type = other DNA
ccatcttccatctgactact

SEQ ID NO: 32 - DNA, 19 bp, synthetic construct
  misc_feature 1..19: note = GluN3B foward
  source 1..19: mol_type = other DNA
cttggctaggttctgagca

SEQ ID NO: 33 - DNA, 20 bp, synthetic construct
  misc_feature 1..20: note = GluN3B reverse
  source 1..20: mol_type = other DNA
gcgtaagctccataccttga

SEQ ID NO: 34 - DNA, 18 bp, synthetic construct
  misc_feature 1..18: note = ADAR1 forward
  source 1..18: mol_type = other DNA
aagactcgggaaacagca

SEQ ID NO: 35 - DNA, 18 bp, synthetic construct
  misc_feature 1..18: note = ADAR1 reverse
  source 1..18: mol_type = other DNA
ccttcttggacagagacg

SEQ ID NO: 36 - DNA, 20 bp, synthetic construct
  misc_feature 1..20: note = ADAR2 forward
  source 1..20: mol_type = other DNA
tgctggactactgtacttca

SEQ ID NO: 37 - DNA, 18 bp, synthetic construct
  misc_feature 1..18: note = ADAR2 reverse
  source 1..18: mol_type = other DNA
ccagagcactttccttcg

SEQ ID NO: 38 - DNA, 18 bp, synthetic construct
  misc_feature 1..18: note = ADAR3 forward
  source 1..18: mol_type = other DNA
ccaggaaagtctccactt

SEQ ID NO: 39 - DNA, 19 bp, synthetic construct
  misc_feature 1..19: note = ADAR3 reverse
  source 1..19: mol_type = other DNA
ccgtgtgctagcctaccat

SEQ ID NO: 40 - DNA, 20 bp, synthetic construct
  misc_feature 1..20: note = REST forward
  source 1..20: mol_type = other DNA
acatgcggactcattcaggt

SEQ ID NO: 41 - DNA, 20 bp, synthetic construct
  misc_feature 1..20: note = REST reverse
  source 1..20: mol_type = other DNA
gaggtttaggcccgttgtga

SEQ ID NO: 42 - DNA, 20 bp, synthetic construct
  misc_feature 1..20: note = RP58 forward
  source 1..20: mol_type = other DNA
gctttcgctctcctgcttga

SEQ ID NO: 43 - DNA, 17 bp, synthetic construct
  misc_feature 1..17: note = RP58 reverse
  source 1..17: mol_type = other DNA
tgtgggaactggcagct

SEQ ID NO: 44 - DNA, 23 bp, synthetic construct
  misc_feature 1..23: note = GluA2 forward for sequencing
  source 1..23: mol_type = other DNA
gaggaatttgaagatggaagaga

SEQ ID NO: 45 - DNA, 22 bp, synthetic construct
  misc_feature 1..22: note = GluA2 reverse for sequencing
  source 1..22: mol_type = other DNA
aggaggagatgatgatgagggt

SEQ ID NO: 46 - DNA, 17 bp, synthetic construct
  misc_feature 1..17: note = Probe for non-editted GluA2
  source 1..17: mol_type = other DNA
catccttgctgcataaa

SEQ ID NO: 47 - DNA, 16 bp, synthetic construct
  misc_feature 1..16: note = Probe for editted GluA2
  source 1..16: mol_type = other DNA
atccttgccgcataaa

SEQ ID NO: 48 - DNA, 31 bp, synthetic construct
  misc_feature 1..31: note = GluA2 forward for detecting Q/R ratio
  source 1..31: mol_type = other DNA
ttgggatttttaatagtctctggttttcctt

SEQ ID NO: 49 - DNA, 22 bp, synthetic construct
  misc_feature 1..22: note = GluA2 reverse for detecting Q/R ratio
  source 1..22: mol_type = other DNA
gaccaaccttggcgaaatatcg

SEQ ID NO: 50 - protein, 883 aa, Homo sapiens; identical to SEQ ID NO: 2

SEQ ID NO: 51 - protein, 906 aa, Homo sapiens; identical to SEQ ID NO: 5

SEQ ID NO: 52 - protein, 894 aa, Homo sapiens; identical to SEQ ID NO: 7